European Patent Specification EP 3 704 271 B1, published January 28, 2026. Title: NEUROKININ ANTAGONISTS AND USES THEREOF. Applicant: California Institute of Technology Anderson, David  J. Zelikowsky, Moriel J. The sequence listing filed with the application follows.

SEQUENCE LISTING (33 sequences)

SEQ ID NO: 1 - protein, 129 aa, Homo sapiens
MKILVALAVFFLVSTQLFAEEIGANDDLNYWSDWYDSDQIKEELPEPFEHLLQRIARRPKPQQFFGLMGKRDADSSIEKQVALLKALYGHGQISHKRHKTDSFVGLMGKRALNSVAYERSAMQNYERRR

SEQ ID NO: 2 - protein, 121 aa, Homo sapiens [sequence omitted]

SEQ ID NO: 3 - protein, 7 aa, Artificial Sequence
  targeting peptide
TLAVPFK

SEQ ID NO: 4 - protein, 7 aa, Artificial Sequence
  targeting peptide
SVSKPFL

SEQ ID NO: 5 - protein, 7 aa, Artificial Sequence
  targeting peptide
FTLTTPK

SEQ ID NO: 6 - protein, 7 aa, Artificial Sequence
  targeting peptide
YTLSQGW

SEQ ID NO: 7 - protein, 7 aa, Artificial Sequence
  targeting peptide
QAVRTSL

SEQ ID NO: 8 - protein, 7 aa, Artificial Sequence
  targeting peptide
LAKERLS

SEQ ID NO: 9 - DNA, 62 bp, Artificial Sequence
  shRNA1 first strand
ccgacgtggttgaagagaacaccgcttcctgtcacggtgttctcttcaaccacgtctttttt

SEQ ID NO: 10 - DNA, 62 bp, Artificial Sequence
  shRNA1 second strand
aaaaaagacgtggttgaagagaacaccgtgacaggaagcggtgttctcttcaaccacgtcgg

SEQ ID NO: 11 - DNA, 62 bp, Artificial Sequence
  shRNA2 first strand
ccgcctcaaccccatagcaattagcttcctgtcactaattgctatggggttgaggctttttt

SEQ ID NO: 12 - DNA, 62 bp, Artificial Sequence
  shRNA2 second strand
aaaaaagcctcaaccccatagcaattagtgacaggaagctaattgctatggggttgaggcgg

SEQ ID NO: 13 - DNA, 40 bp, Artificial Sequence
  shRNA1 Forward
aaccacgtcttttttaattctagttattaatagtaatcaa

SEQ ID NO: 14 - DNA, 33 bp, Artificial Sequence
  shRNA1 Reverse
cttcaaccacgtcggctgggaaagagtggtctc

SEQ ID NO: 15 - DNA, 40 bp, Artificial Sequence
  shRNA2 Forward
ggttgaggcttttttaattctagttattaatagtaatcaa

SEQ ID NO: 16 - DNA, 33 bp, Artificial Sequence
  shRNA2 Reverse
atggggttgaggcggctgggaaagagtggtctc

SEQ ID NO: 17 - DNA, 18 bp, Artificial Sequence
  mCherry  Forward
ctcctcgcccttgctcac

SEQ ID NO: 18 - DNA, 24 bp, Artificial Sequence
  mCherry  Reverse
ggcgcgccataacttcgtataatg

SEQ ID NO: 19 - DNA, 48 bp, Artificial Sequence
  pAAV-GFP Forward
cctggacctatggtgagcaagggcgaggagctgttcaccggggtggtg

SEQ ID NO: 20 - DNA, 55 bp, Artificial Sequence
  pAAV-GFP  Reverse
agcatacattatacgaagttatggcgcgccctacttgagctcgagatctgagtac

SEQ ID NO: 21 - DNA, 1274 bp, Artificial Sequence
  Tac2-P2A-mCherry
gctagcgccaccatgaggagcgccatgctgtttgcggctgtcctcgccctcagcttggcttggaccttcggggctgtgtgtgaggagccacaggggcagggagggaggctcagtaaggactctgatctctatcagctgcctccgtccctgcttcggagactctacgacagccgccctgtctctctggaaggattgctgaaagtgctgagcaaggcttgcgtgggaccaaaggagacatcacttccacagaaacgtgacatgcacgacttctttgtgggacttatgggcaagaggaacagccaaccagacactcccaccgacgtggttgaagagaacacccccagctttggcatcctcaaaggaagcggagctactaacttcagcctgctgaagcaggctggagacgtggaggagaaccctggacctatggtgagcaagggcgaggaggataacatggccatcatcaaggagttcatgcgcttcaaggtgcacatggagggctccgtgaacggccacgagttcgagatcgagggcgagggcgagggccgcccctacgagggcacccagaccgccaagctgaaggtgaccaagggtggccccctgcccttcgcctgggacatcctgtcccctcagttcatgtacggctccaaggcctacgtgaagcaccccgccgacatccccgactacttgaagctgtccttccccgagggcttcaagtgggagcgcgtgatgaacttcgaggacggcggcgtggtgaccgtgaccaggactcctccctgcaggacggcgagttcatctacaaggtgaagctgcgcggcaccaacttcccctccgacggccccgtaatgcagaagaagaccatgggctgggaggcctcctccgagcggatgtaccccgaggacggcgccctgaagggcgagatcaagcagaggctgaagctgaaggacggcggccactacgacgctgaggtcaagaccacctacaaggccaagaagcccgtgcagctgcccggcgcctacaacgtcaacatcaagttggacatcacctcccacaacgaggactacaccatcgtggaacagtacgaacgcgccgagggccgccactccaccggcggcatggacgagctgtacaagtaaggcgcgccataacttcgtataatgtatgctatacgaagttattaagaggtttcatattgctaatagcagctacaatccagctaccattctgcataacttcgtataaagtatcctatacgaagttattccggagtcgac

SEQ ID NO: 22 - DNA, 18 bp, Artificial Sequence
  Digoxigenin-labeled Tac2  Forward
agccagctccctgatcct

SEQ ID NO: 23 - DNA, 18 bp, Artificial Sequence
  Digoxigenin-labeled Tac2  Reverse
ttgctatggggttgaggc

SEQ ID NO: 24 - DNA, 20 bp, Artificial Sequence
  Tac1 Forward
gatgaaggagctgtccaagc

SEQ ID NO: 25 - DNA, 20 bp, Artificial Sequence
  Tac1  Reverse
tcacgaaacaggaaacatgc

SEQ ID NO: 26 - DNA, 19 bp, Artificial Sequence
  Tac2  Forward
gccatgctgtttgcggctg

SEQ ID NO: 27 - DNA, 20 bp, Artificial Sequence
  Tac2  Reverse
ccttgctcagcactttcagc

SEQ ID NO: 28 - DNA, 19 bp, Artificial Sequence
  GAPDH Forward
tgaagcaggcatctgaggg

SEQ ID NO: 29 - DNA, 20 bp, Artificial Sequence
  GAPDH  Reverse
cgaaggtggaagagtgggag

SEQ ID NO: 30 - DNA, 20 bp, Artificial Sequence
  18s Forward
gcaattattccccatgaacg

SEQ ID NO: 31 - DNA, 20 bp, Artificial Sequence
  18s Reverse
gggacttaatcaacgcaagc

SEQ ID NO: 32 - DNA, 8514 bp, Homo sapiens
cacgcaagcgaaaggagaggaggcggctaattaaatattgagcagaaagtcgcgtggggagaatgtcacgtgggtctggaggctcaaggaggctgggataaataccgcaaggcactgagcaggcgaaagagcgcgctcggacctccttcccggcggcagctaccgagagtgcggagcgaccagcgtgcgctcggaggaaccagagaaactcagcaccccgcgggactgtccgtcgcagtaagtgcccgcgcggtgctggccgcggctgcccgggtcaccccgccccgcatctgtccgaggtggccgcgctgggggcgccgctgcggcgagggacagtggggagactggcttcccaaacgccaacgcccctctttgtcttccacctgcagagtttcctggtttgaaggtgtgggttggtgggttagggggctgggggagttgggattcagggagaagagggttggagaatctttgggacgcgattctctcgcctaaccggtacaggtgagacttcagtccttatgtttttgatcttggttcatccgttgtggggcagaaaattctgttgctttaactcttggataaccacccctaatagatacattatttctctctttggtgtcttctcctcctaccccttcccagaaatccaacatgaaaatcctcgtggccttggcagtcttttttcttgtctccactcagctgtttgcagaagaaataggagccaatgatgatctgaattactggtccgactggtacgacagcgaccagatcaaggtgaggccccttcccaggacggcccgcacccttcttcctgggctcgggagctgtcaccttcccacgcaacagcaccctagttaacgtggcacgcaccgccaccacggaaagaggcagcggttgcgtgcgagaggatggaaaggggcactatttcccgggttccccacgggattttgtgcccacgattcaagtttcttcccgagggctgcaccgtccggcccaggaactccctgcagtagggatgccctcccggatgagcccgagatcctcacaaggcgggaaatctcgtaagatttcatcccccaggacctgggatttcgggggctccggtccagctgcactgccctagcgtctgggcacgggcagaggagggcgcctgggtcgcgggcagcagcgggcacacgcgcgagctgcagggggattggagggccggaggctggagggaagttaatttcctgccttcacgtttgttttgcggacctgaggatgtagcttgaagtctccctttagaaactcgtaggctacaggcgctggggagcgcgcctcggaaaaacggtgaaagtcgtctgtaaagcgttgtcacccttccccaccggagccccagccccagatcccacacacctgtgtgcatttagggcggtgaggactctacaaagccggcaccgagacaagacaaagtcaggtggcggcgcagcagatgagggaaggtccccgggctgggaggaaagagcggaaagcgctcgaagcttgaagacgccgagccagctgctaactcgccctggcaggcttgcggggggcgggacgcgagttcggcggggaggggcgcagagaggcagcgcctcgggagggaccccgctcagcccgagcgtggggaaggccgcctccccacgcctcggggccggagtacagcggggggaagggctcgggttgctgggtgcctcgctctggttgccttacacgccctttgtccgtgcttttgtctcccaggaggaactgccggagccctttgagcatcttctgcagagaatcgcccggagacccaagcctcagcagttctttggattaatgggcaaacgggatgctggtgagataggcgaccgtccctaggtgtcttgggcagcccgccctgtctgctcactccttcctggagtaccccagggtctctcgctctgaatagagatttccactccaagaggggtgtaattccccaggcgcgacattggcccacaccgcactaaggcacgcacgggcccgcggggggagggaaagatctggttcgcatgcctcactgtattcgagtgaagcgctcccttgactaaagatccaaactgacaaagggaaggcacgggcctccaggggtagtactgcggatgatccaagtgcatgtggaagaggattttatagcattccctgaggtgagagtacatttgtcttgggatagaaatatcgtttccttgaattcatcgcacggtcagtggaacatgtagttaatgacaattcgtctcttgtcagattcctcaattgaaaaacaagtggccctgttaaaggctctttatggtaaacattcctataaatctttattttactattgtgaaagcacatgtaggaaagtgaaataaaatcttttatgggctgaaatacaagatctgggtcatgcctgtttaataaagagatggatttgcgcactctctctcggtttctctctctctctgtcactctctctgtctctctctctctgtcactctctctcagtctctctctctctctttctctctctctctcagtgggtggccagccttgaaggtgggatgtgttacagtcttatagttaataagaggcctcagaagtctcatagtcctaggtttgaatcccatagaaggcacttaataaaaattccatttgtttgtttaaatatttagtttttatgattaataatttgtttagcatttatggttctgctttattcctcaggataatatatagatagaaaatgttacatattttgagaatcaaattattttataaaagatataatgtagcatctttaaaaacaaatctatatgtgtttgctaattttatctttcttctaggacatggccagatctctcacaaaagtaagttcaaaattattttgacatttatcaaatttaaatgtaaaattatattgaatttcactttatttatcttaccttattttctgtcatgactctagggcttaatatgtttaatgaagacaatataagaatgggggagattcatattacatccagaatatggttgtttagacatattgtacttagcaaagagatgcattatattaaaaaagaaaaaaatgtcttttaagtcccttcaattgttagttttagagaagaatttcaatcctaggattagaaatctaccatacatatttcttcccagccacccaccccctaagcttactttcactgtaaacaaacaaacaaacaaacacgaaacccccacaagcatttataggcatctcctaactcattttagtatgcttggtccaataatgatgtcatttattagggtcatccagcagccaattaaatggaatgagtgagtgaacatgagtagagaatccatactaaaaatgaagacggtagagatgcagttttttaatcccctaattgaatgggaaaactcgatcagtaaaacatttcttagggcagcaaagatggcaaaattgtggtatgtgaaggtcattaaatttgtttctcagttaatggaaccggagttgacaagaagtggaaagggtctatcttcatcgtattgtccactcacctattgtaccctgtcatggatttggttcattgggtggcagagcaggccacattaacgtagcagctctattctcaactattaaaataaaaaccaagagaaattctctcactagcattaaaatagtaacctttccaaagagttcatctttgaaaaataaatagtattcatatttactttctaaggatttgactttgaagagaattatatataaaaattctatgtaataaaaaatgtactctgttcatgtgaaaactaataaacttttctgaaaggagtatcttttaatatccaataaaataaaaacagtgaccttttagaagattataatcatcaaggaaaggaatctggtttaattaaggtctacttgctgagaagtacaacttattaataacacaaggaattatgcttggatatttcactctcacacaaatgtgaaattgacttcctaaaaaatcaaacctagctcaaataacaatattttatataaaatattttagacccttacataacagataaaatatatgaatagagagtgcttgctaatattaaatatagaattaagaaaagtggtttcattgtattgttttagtgtaatttataaaacttttaaggaatctttatttcttcagtctcaccaaaacttgaagtagatagatatttattatacagacatatattcagaagcttgctttgttctggttataatagtttgtttcctcaaagatatacatattaaaatacccctaaatgtatttttccaggacataaaacagattcctttgttggactaatgggcaaaagagctttaaattctggtatgtatgaaattatgactgaaaatagacagtatctcaaatctatttctattttttctaagacatagttttaaaatattaaaaaggagtggtagatataaaaatgagtattatggtggaaaaatttaattgttgtacttgtaaccacaaatggatttatagctggttaagctaatactaccacagtatctgtctatttctctccaatcaccattcttaccagtgtctgccccatttaatcattaccaacctgaatctttgggttagtgctatattctttcctatagatctgttaaataagccgtgtttaaccttactgaactaagggggagtggggagtgcagggaagaatgagggtgattttcacttgttatcaaagtaatttgaaagttttacaagacattacatttggcgatcttccaatacaaaaataaattcacaaaacaaattctttatgcaaattaatcactttttatgaagttgtagaaattcaaaatctaaacatcctgatggatgttggagaggacaaaagtgatacggtttattccagtactttcaaaaaggaacacaattaaatatccttgagtgttataaattggttctggctataaactccttagagagaaaggatgccacaattctcattttaattctgaacaactttttcgtatgatataaaggctgcaggtttccttctcttcaatttccatcttctttgtaaataccacgtacatatatctgaaaaccattattagttaactcattcatcacactgatttcaatgtaaataacccctagatcattttaatagaagctcactttttgttaagaccttatagctcttacctctagggcttcttggaaaagctattcaaattctattttgccttcagtgaaaatagaattaaaatactaaatacgttattaattataaagtaatcagcagctgtcttacccatttagaatatttccagtttctagacaatctataagatgtgctggcttaatccttaattatctggatcctaggaaaaataattatcctagtgttttttaatggagatttttttctttattgtgaaatgtaagacttgggtacattaaataaaaccactttctgtggggcaaaaatcaaaacgcgcaatagaaaaaaaaagttaacacaatctgggctacggcagaagccagagaatatattcatataattgaaaagttctaagtgtttcataattgaccttttgatacaaaatttccaataaatctggaatttgaagttcttggtgaagtccacaggacttcctagtgttcttattgggtccccactttctatttagacactacctttgcatcttctcaccagtcattttgggctgccgaagtgtaaaagtgtaagaaattatcaatgtgccttaatgaaaaacttgtaattgttttattaatatgtattatcttcccacttttggaaatgaaatataaatttaaaccacaatggcttttatttgtaccaatacatactagtcctcacttaattgtagttttcttgataatcatattagtcatcaactttccatttccagaattgatataggtttcagaacatgcttaactttacaaatgtagatattgtacaagttagaacagattaaatacaattaaatgtacttaaaataataacataattttaagtagtgataaaaatcactgtagtgaatcaggatcaatttataactaaatctttgttcctccattttagttaaggaaatataaataggtgaaatgtggaaaaaaatgtgatatgatccacagtcaatcagggatctttttatgtacctcattgaggcaaggttatcatagccttaatctatagccctctgatctttacccactcatggtcagggacccctttgacaatctgataaatctagatagatgccctttcccagagaaaccctcatcagctcatacactcaaaaatttatatcaggcttcagagggttcaaagaccaggtaagaaactctgcttccatgtaagaggacattatgttccagctaaatcactgtctgtctttagttggtttacattagctttcatctaatttctctgaggaatagagtcatgttacctaaagcttgtcagagactgaacttgggccattcatcctgttcctaatataatcaaaccagaatgagaaataaactgtttccttccctcacgcctgtccagtgttggctcagactgttctgcctcacaagtgcatacttaattgatgtaaaatatgcagcttattgttaaccgcacttaaaggatagctgggtgtttaagaccagtattaaaagagggaagtgataatactggtgcctttacctgtcttctctgtcagcaaatcttctcactgaggaaactgtttagagtagcacttattattcctacagatccttcacagatctttctactctttctgtttacattcagtattttatacaggccatactgaatttcaaaaagcatagtagttccactataccatacgtctaagtctataaggtattcgttaaggatgaaaaatatcccaaaatacttttattgcaacagtctgatttttacccctttgtggttacagatccctttgaaattatatataataaatataatataatataatatacaattttggcatttttttgtccagataatcaatgtatttaaattacttgctagctatatgttaaatacctttggaagcaataattaatgcttcacaggccattaaggtgctagtgaaaagttaaacagtatggtatttagatggctcaactgacttacctatggtaaatgggctgtttttagtcttgagggcagtccatcactgggaggtatccacaaggtaggaagagacccctacacaattagatgccccttgaacaaagatcagcaaacttttcctgaaaagaaacagattataaatattttaggctttgtgagccatgtaatctctgttgcaactacccaaatctgttattttaggccaaagcagccatagacaatatgtaaatgaatgagtgtgtctgtattcctataaacctctttacaagaacaaatggtattctagatttggcccatggtctctgctagaataaaagtcccacatttggtttttatcctactagtattcctggttattttaggcattgtcctttctagaattcactatgggtatctgccactgcttgagaaagctgctgagaatcaacactgcaatatattgtggaaatatgctttgggggcaccaagtatatgatgaatgatgaatgaaaccgagttctgtggttagatcatttccaatcagaatagagactgaggcaggattggaagatgtgcagataacattcttagaaatacttctgtagagggaaaatgtcattatgagtttaaaataaattactatatgccctgaactttagttgtgtaactccctcagtgaattcacttaaaaaacactttatctcttctttgttttcagtggcttatgaaaggagtgcaatgcagaattatgaaagaagacgttaataaactacctaacattatttattcagcttcatttgtgtcaatgggcaatgacaggtaaattaagacatgcactatgaggaataattatttatttaataacaattgtttggggttgaaaattcaaaaagtgtttatttttcatattgtgccaatatgtattgtaaacatgtgttttaattccaatatgatgactcccttaaaatagaaataagtggttatttctcaacaaagcacagtgttaaatgaaattgtaaaacctgtcaatgatacagtccctaaagaaaaaaaatcattgctttgaagcagttgtgtcagctactgcggaaaaggaaggaaactcctgacagtcttgtgcttttcctatttgttttcatggtgaaaatgtactgagattttggtattacactgtatttgtatctctgaagcatgtttcatgttttgtgactatatagagatgtttttaaaagtttcaatgtgattctaatgtcttcatttcattgtatgatgtgttgtgatagctaacattttaaataaaagaaaaaatatcttgaa

SEQ ID NO: 33 - DNA, 6564 bp, Homo sapiens
ctttatcagggagctgggactgagtgactgcagccttcctagatcccctccactcggtttctctctttgcaggagcaccggcagcaccagtgtgtgaggggagcaggcagcggtcctagccagttccttgatcctgccagaccacccagcccccggcacagagctgctccacaggtaggcaagtgggagaatgctggatggaccagagctggcaccaggggacaggagccagcgtcaggagggaataaagcagatggcagcctctgataggggagcaggggactgggaaggtgagcacaaagcacctgtagggccgagagctggttggtgtttggagcctgtggctacagactcattctttcataccagaaagtttttgcctaagtcttgggattatctagtactggaaaatagcatccaggatccctcctccagctgactgaggaaacagaccagtccatgtcctacaaatctatcatctttcttgggagctagagtcctcctggcaccactatagcattgcacatctcctggggagatatctgatggggtagcagggaaactaagcccaagggctgtacccccttctcagaaatactttccaccctctctccagaccagggcttggacagtggagttgggggctggggaagcagggtcaagccaagctgctggtaatgaatgtctcttgtgtcttcacccatgctgtatcttcctcttctctcctttacctgagtcctgtccctttgctctcccaggcaccatgaggatcatgctgctattcacagccatcctggccttcagcctagctcagagctttggggctgtctgtaaggagccacaggaggaggtggttcctggcgggggccgcagcaaggtaagtctcccctggcagagtactggggacatcacgggaacttgggactctgcctgtctggacagctgtagtgaggaaactggggtgggggggttgtccgtcagagggcattttgcctccctttggatttctttgtttctctggtcctttcatgttcccactgtctccaggtgtgtttgtgtctctgtatctctgcatgtctttgacaccttgtacataaaaggtgccctacaaatatgttgtttggtgggttgattgatgggagacttggtgattggatggtactgtgaggggtgagctagggtggtctaaggctctctatagtctacctcaggtccctttgcaagggacagatctcttctatttcctggatggtatgaaacagtcagaatttctttcccaaatggttatttgtgtgctattttacctatcagttatgtgtattgttttattttcaaaatgcaaataaattcccttatcttttgctcatccacccccagtaacctcaggtgcttctaagatcccaaccccttccttcttctcttttctcccttgcccgcctctatcctctgcttagtcaggataggaaaacaacaacagcaaaaaaaccagattgagcctcgatttccacagttcctttacgaaaaagaataggaattgtcagggtaggggtacagggggaggatagggaggaagtcttttcaaggttttgaaatgacagcaattacatcggtacaaatgcttttaagatgattgcgggtgggacttattacaaattcaatgtgtgaagtttaactgcctcttcagctcaaatctgttcagcatctcattataggaggtgggcagagtattcaacaatttgggaaaagtggctgcctgaacaccacatgctgggccaagggagttatcaccagggcagccttgcaggtggcagcagttgtgccatatccaaaaggccagaaccgttaaaaaaaaaaacacccaggggagtgccaagtatgggctggacaccgtttggagccacaaagttccagcccaggatagttagagtatctgagttcttctgagacaaacttgtttcaagaccttggccaatgagatgtcccctctgcccctcttggtcaatgaatgagagggattgccatcctaccccttctccttgagagtctgtgaggatgagggaaattggggcaggaagagggtagtacataggtgtgcctaggcaactgggttggtatgtgtgggggtgtgttctgtgtaaatgcacttctgtgtgtgcacaacagccgaaggatgcctgggttctggaaagagaggcgctgctgagacttgagatttgagatgaaaatctccagccatgatcattgttattgtctctctgcagctgcaattaactggctgtgtggtgtgtgcccaccaccctgctgtacgcaagttgctaaaaaaaaaaaaaaaatcacagggacaatcaagagcccgtgctgggcaacagctctagaacttgggattcagttgtggagagaagaagacgtgccttctgagcatgttgccttcctggaattctagacctagggccaaaagggagagggagagaaaactagaggcggaaagccatggagaatagagaaagaggtggtggaaaacagggagagaaacatccatggacatcgtgcagagtgggggaatcacaggtgcagatgtgtgcctccaatctcaccatgcatgtgaatcacctggggggctgcttaaaatgcagattctgtctcaggaggtctggggtaggaacaagagtctgcatttctaacaggctctgtgtagtgctggtgttgctgttggtccacaggtcactcctggagcacctacttctcgtccagtgtgaaccagaggaaactctgaaagaaatagggtgtcggattcaggatgggctcaggaagaggctgtttcttgtgggaaaaggatgagtggatccgggtgggagcctcctgcctcacccctctttgtttcttccctagagggatccagatctctaccagctgctccagagactcttcaaaagccactcatctctggagggattgctcaaagccctgagccaggctagcacaggtaggaggcggccctaggggagaggggaatgaggggcaggattctgaagataagaggcctgggagatcctttcagatgggagagagatgggggatagcttagtgaatcggtgagggttgtgatctgaaccccgctctcatcactttccaacttcactccccatttagacatctgttcttggtttcacagatcctaaggaatcaacatctcccgagaaacgtaagtaccctcttctccctccctatctcttgccacttgcccagagctctgtggggcattgggcccaggggccattttgtccagccccttctcacctggtacaaacaatatgccagctcccactgctcagccaacctttcctgaaagggagaggccatccagaactaggaggaagctggtgtgaggggcatggtgggctctccctctgctggctggtccttggaaaacaaggggatctcttcgtggccctgaaaattccaaatcaggcacctgctagagcagaaaattcttgaaatgtggaggaaggaaaggtgagcagagagagtgggtttaggggaggcacttgctaactgtgaggagtcatgctttgacaagaaaaaggaacagagaccagaaacccagtctcagaagtgttgacccatgtctggggagatgcttcactttctcatcatcactgctgacaatgttggcccttttctgcaggtgacatgcatgacttctttgtgggacttatgggcaagaggagcgtccagccaggtaggagtgtgtggaggtacagtggaagggcttagggtactggcagagtatgacagaagtcacgtgcctcatatttgtcaccagagggaaagacaggacctttcttaccttcagtgagggttcctcggccccttcatcccaatcagcttggatccacaggaaagtcttccctgggaacagaggagcagagacctttataaggtagtcctgttgcagctgggaggaaggatagggagactctgcttccaccccagtctcccaactctgtctttgaacactgcccgtcatagccagccctttgctgttggatcagggtgtagttcacattcagaaagatccctcttacttacactgttcgctttaccctagactctcctacggatgtgaatcaagagaacgtccccagctttggcatcctcaagtatcccccgagagcagaatagggtaaggattgttcattagagaggggagaggggactggggagggggctgtgggggttgccagctgtgcatttcctcccatgctacaggtattaaagctcatagatttgccctgaaatacactgccaatgcccagcacactgtcggccaaacacaaagacacttagaggcacgtgtgtttgtacacatcccccgtctttcatctctttcctctggatcatggacggcagctgactattgagcaggagtgagtgttgggagatgaggagagaggggcttccccgatgggcaatttctgttgtttggacttcattcttttgtaatctatgcaaaaagatggagaaattattatctgataattacaaataccacaaccaattcacaggcaagcatttgcctcccaggcaggctgagcctttcaaatcactcagaatcctgggttacggggcccagaaggtagtcatacacaaggatgattcaggaagaaatgcaaggaactctgaaatctaatggggattagcaggaaaccatatctgaatctctctttagcataatgaataagaacaatggcctgaatgtgaatcctggatctgccactctatctgtatctttttggccaaggtacatatcctcctgtgcttcagtttcctcatctgaaaaatgaaagtgataatagtatctcacagggttgtggttttgaggattgagtataggtaaagtgttcagaacagtgccgggtgcacagtgctgtgtgccaattttatgataattgtcccagtttgggaggtatgggggatgtcctaatgtttcccctgactggctctgtctggaccccaggcctgagtgggctgacaaattcctcacttggtatgcgagtgtaagagtcccccagggaagtgtctagtcaaaacacgaaccttccgccttgacactgtcttcccacacacagcaagagcagctccaccaatggctttcttttcactagcttccaaagaattggggtggagggagtgaaaaggagagggagagagattgggaaggctcgtaatcatggagagcctcctgcttttctctctgtgtccctgttacccatactcactggtctcaaggtggcacgcccaagacccaaggagctggtgcttgatgatgctgcctgtgcatgaattcctgggaccagagactgagtctggccccccatttagtgttgggtgagagggcacaaagagctataataactgtaacttgctgattacatggtagttactgtatcattttgctctcattagatggttatttcagtcctgccgacggccagataattatacgagcagctatatctggatgacatactctgctccagcgttatgcactggccataaagataattacagtgcaattttgctatagtattttatacaaatggcaaaaacaagtgcattgtggaaatctacttttaatgcttgtttgtgcatccaggctctttcagagggacccataattgcagctttcataatcttaccattgagggagcattcccaacctgttaggtgtcaggcagaataggacataaggtttctgggagctggcatttaaagattagatgagatggatcaacacagatcattgtgtcatctgatttcattcatgtgaaactgtaagtaatccctgggcctgtgcttcctctgggaggtttctgggaagaggaggaactggataaggcagggggagcattcatagtagggcaccttgggcagggctgtgtgtgtgtctggctcatggtggtgctaggatggcatgaacttggttcctacatctttggtccacatgggccccactggccatgcacacaggtgtgtagagtaatgtaaatatggcagctgggaaggtgcaagtacctgcggctaggagagttccatcctcaggcccaaagcctggagggcaggctgagggtcaagacttgttctttcctctctcacagacgcctctccccttctctcctgctgccacagcaggttttcagtgggacttttttacaggatataagatgtgatttcagtgtttttttttgttttgttttgttttttgtcctcagtactccacttccggactcctggactgcattaggaagacctctttccctgtcccaatccccaggtgcgcacgctcctgttaccctttctcttccctgttcttgtaacattcttgtgctttgactccttctccatcttttctacctgaccctggtgtggaaactgcatagtgaatatccccaaccccaatgggcattgactgtagaataccctagagttcctgtagtgtcctacattaaaaatataatgtctctctctattcctcaacaataaaggatttttgcatatgaatga